European Patent Application EP 4 332 214 A1, published March 6, 2024. Title: Novel Lactobacillus fermentum ATG-V5, and composition for enhancing immunity comprising thereof. Applicant: AtoGen. The sequence listing filed with the application follows.

SEQUENCE LISTING (1 sequence)

SEQ ID NO: 1 - RNA, 1448 nt, Artificial Sequence
  16S rRNA of Limosilactobacillus fermentum ATG-V5
atgcagtcgaacgcgttggcccaattgattgatggtgcttgcacctgattgattttggtcgccaacgagtggcggacgggtgagtaacacgtaggtaacctgcccagaagcgggggacaacatttggaaacagatgctaataccgcataacagcgttgttcgcatgaacaacgcttaaaagatggcttctcgctatcacttctggatggacctgcggtgcattagcttgttggtggggtaacggcctaccaaggcgatgatgcatagccgagttgagagactgatcggccacaatgggactgagacacggcccatactcctacgggaggcagcagtagggaatcttccacaatgggcgcaagcctgatggagcaacaccgcgtgagtgaagaagggtttcggctcgtaaagctctgttgttaaagaagaacacgtatgagagtaactgttcatacgttgacggtatttaaccagaaagtcacggctaactacgtgccagcagccgcggtaatacgtaggtggcaagcgttatccggatttattgggcgtaaagagagtgcaggcggttttctaagtctgatgtgaaagccttcggcttaaccggagaagtgcatcggaaactggataacttgagtgcagaagagggtagtggaactccatgtgtagcggtggaatgcgtagatatatggaagaacaccagtggcgaaggcggctacctggtctgcaactgacgctgagactcgaaagcatgggtagcgaacaggattagataccctggtagtccatgccgtaaacgatgagtgctaggtgttggagggtttccgcccttcagtgccggagctaacgcattaagcactccgcctggggagtacgaccgcaaggttgaaactcaaaggaattgacgggggcccgcacaagcggtggagcatgtggtttaattcgaagctacgcgaagaaccttaccaggtcttgacatcttgcgccaaccctagagatagggcgtttccttcgggaacgcaatgacaggtggtgcatggtcgtcgtcagctcgtgtcgtgagatgttgggttaagtcccgcaacgagcgcaacccttgttactagttgccagcattaagttgggcactctagtgagactgccggtgacaaaccggaggaaggtggggacgacgtcagatcatcatgccccttatgacctgggctacacacgtgctacaatggacggtacaacgagtcgcgaactcgcgagggcaagcaaatctcttaaaaccgttctcagttcggactgcaggctgcaactcgcctgcacgaagtcggaatcgctagtaatcgcggatcagcatgccgcggtgaatacgttcccgggccttgtacacaccgcccgtcacaccatgagagtttgtaacacccaaagtcggtggggtaaccttttaggagccagccgcctaa